European Patent Application EP 4 566 632 A1, published June 11, 2025. Title: MSLN抗体药物偶联物. Applicant: 诺纳生物（苏州）有限公司. The sequence listing filed with the application follows.

SEQUENCE LISTING (79 sequences)

SEQ ID NO: 1 - protein, 25 aa, synthetic construct
  source 1..25: note = 945
QVQLVESGGGVVQPGRSLRLSCAAS

SEQ ID NO: 2 - protein, 10 aa, synthetic construct
  source 1..10: note = HCDR1
GFTFSSDGMN

SEQ ID NO: 3 - protein, 14 aa, synthetic construct
  source 1..14: note = HFWR2
WVRQAPGKGLEWVA

SEQ ID NO: 4 - protein, 17 aa, synthetic construct
  source 1..17: note = HCDR2
VIWNDGSNKYYADSVKG

SEQ ID NO: 5 - protein, 32 aa, synthetic construct
  source 1..32: note = HFWR3
RFTISRDNSKNTLYLQMNSLRAEDTAVYYCAR

SEQ ID NO: 6 - protein, 10 aa, synthetic construct
  source 1..10: note = HCDR3
DRGPLWPLDY

SEQ ID NO: 7 - protein, 11 aa, synthetic construct
  source 1..11: note = HFWR4
WGQGTLVTVSS

SEQ ID NO: 8 - protein, 23 aa, synthetic construct
DIQMTQSPSTLSASVGDRVTITC

SEQ ID NO: 9 - protein, 11 aa, synthetic construct
  source 1..11: note = LCDR1
RASQSISRWLA

SEQ ID NO: 10 - protein, 15 aa, synthetic construct
  source 1..15: note = LFWR2
WYQQKPGKAPKLLIY

SEQ ID NO: 11 - protein, 7 aa, synthetic construct
  source 1..7: note = LCDR2
KASSLES

SEQ ID NO: 12 - protein, 32 aa, synthetic construct
  source 1..32: note = LFWR3
GVPSRFSGSGSGTEFTLTISNLQPDDFATFYC

SEQ ID NO: 13 - protein, 9 aa, synthetic construct
  source 1..9: note = LCDR3
QQYNSYSRT

SEQ ID NO: 14 - protein, 10 aa, synthetic construct
  source 1..10: note = LFWR4
FGQGTKVEIK

SEQ ID NO: 15 - protein, 10 aa, synthetic construct
  source 1..10: note = HCDR1
GFTFSSDAMN

SEQ ID NO: 16 - protein, 17 aa, synthetic construct
  source 1..17: note = HCDR2
VIWNEGSNKYYADSVKG

SEQ ID NO: 17 - protein, 17 aa, synthetic construct
  source 1..17: note = HCDR2
VIWNDASNKYYADSVKG

SEQ ID NO: 18 - protein, 9 aa, synthetic construct
  source 1..9: note = LCDR3
QQYSSYSRT

SEQ ID NO: 19 - protein, 9 aa, synthetic construct
  source 1..9: note = LCDR3
QQYNAYSRT

SEQ ID NO: 20 - protein, 9 aa, synthetic construct
  source 1..9: note = LCDR3
QQYQSYSRT

SEQ ID NO: 21 - protein, 9 aa, synthetic construct
  source 1..9: note = LCDR3
QQYNTYSRT

SEQ ID NO: 22 - protein, 9 aa, synthetic construct
  source 1..9: note = LCDR3
QQYTSYSRT

SEQ ID NO: 23 - protein, 9 aa, synthetic construct
  source 1..9: note = LCDR3
QQYASYSRT

SEQ ID NO: 24 - protein, 119 aa, synthetic construct
  source 1..119: note = VH
QVQLVESGGGVVQPGRSLRLSCAASGFTFSSDGMNWVRQAPGKGLEWVAVIWNDGSNKYYADSVKGRFTISRDNSKNTLYLQMNSLRAEDTAVYYCARDRGPLWPLDYWGQGTLVTVSS

SEQ ID NO: 25 - protein, 119 aa, synthetic construct
  source 1..119: note = VH
QVQLVESGGGVVQPGRSLRLSCAASGFTFSSDAMNWVRQAPGKGLEWVAVIWNEGSNKYYADSVKGRFTISRDNSKNTLYLQMNSLRAEDTAVYYCARDRGPLWPLDYWGQGTLVTVSS

SEQ ID NO: 26 - protein, 119 aa, synthetic construct
  source 1..119: note = VH
QVQLVESGGGVVQPGRSLRLSCAASGFTFSSDAMNWVRQAPGKGLEWVAVIWNDASNKYYADSVKGRFTISRDNSKNTLYLQMNSLRAEDTAVYYCARDRGPLWPLDYWGQGTLVTVSS

SEQ ID NO: 27 - protein, 107 aa, synthetic construct
  source 1..107: note = VL
DIQMTQSPSTLSASVGDRVTITCRASQSISRWLAWYQQKPGKAPKLLIYKASSLESGVPSRFSGSGSGTEFTLTISNLQPDDFATFYCQQYNSYSRTFGQGTKVEIK

SEQ ID NO: 28 - protein, 107 aa, synthetic construct
  source 1..107: note = VL
DIQMTQSPSTLSASVGDRVTITCRASQSISRWLAWYQQKPGKAPKLLIYKASSLESGVPSRFSGSGSGTEFTLTISNLQPDDFATFYCQQYSSYSRTFGQGTKVEIK

SEQ ID NO: 29 - protein, 107 aa, synthetic construct
  source 1..107: note = VL
DIQMTQSPSTLSASVGDRVTITCRASQSISRWLAWYQQKPGKAPKLLIYKASSLESGVPSRFSGSGSGTEFTLTISNLQPDDFATFYCQQYNAYSRTFGQGTKVEIK

SEQ ID NO: 30 - protein, 107 aa, synthetic construct
  source 1..107: note = VL
DIQMTQSPSTLSASVGDRVTITCRASQSISRWLAWYQQKPGKAPKLLIYKASSLESGVPSRFSGSGSGTEFTLTISNLQPDDFATFYCQQYQSYSRTFGQGTKVEIK

SEQ ID NO: 31 - protein, 107 aa, synthetic construct
  source 1..107: note = VL
DIQMTQSPSTLSASVGDRVTITCRASQSISRWLAWYQQKPGKAPKLLIYKASSLESGVPSRFSGSGSGTEFTLTISNLQPDDFATFYCQQYNTYSRTFGQGTKVEIK

SEQ ID NO: 32 - protein, 107 aa, synthetic construct
  source 1..107: note = VL
DIQMTQSPSTLSASVGDRVTITCRASQSISRWLAWYQQKPGKAPKLLIYKASSLESGVPSRFSGSGSGTEFTLTISNLQPDDFATFYCQQYTSYSRTFGQGTKVEIK

SEQ ID NO: 33 - protein, 107 aa, synthetic construct
  source 1..107: note = VL
DIQMTQSPSTLSASVGDRVTITCRASQSISRWLAWYQQKPGKAPKLLIYKASSLESGVPSRFSGSGSGTEFTLTISNLQPDDFATFYCQQYASYSRTFGQGTKVEIK

SEQ ID NO: 34 - protein, 449 aa, synthetic construct
  source 1..449: note = HC
QVQLVESGGGVVQPGRSLRLSCAASGFTFSSDGMNWVRQAPGKGLEWVAVIWNDGSNKYYADSVKGRFTISRDNSKNTLYLQMNSLRAEDTAVYYCARDRGPLWPLDYWGQGTLVTVSSASTKGPSVFPLAPSSKSTSGGTAALGCLVKDYFPEPVTVSWNSGALTSGVHTFPAVLQSSGLYSLSSVVTVPSSSLGTQTYICNVNHKPSNTKVDKKVEPKSCDKTHTCPPCPAPELLGGPSVFLFPPKPKDTLMISRTPEVTCVVVDVSHEDPEVKFNWYVDGVEVHNAKTKPREEQYNSTYRVVSVLTVLHQDWLNGKEYKCKVSNKALPAPIEKTISKAKGQPREPQVYTLPPSREEMTKNQVSLTCLVKGFYPSDIAVEWESNGQPENNYKTTPPVLDSDGSFFLYSKLTVDKSRWQQGNVFSCSVMHEALHNHYTQKSLSLSPGK

SEQ ID NO: 35 - protein, 449 aa, synthetic construct
  source 1..449: note = HC
QVQLVESGGGVVQPGRSLRLSCAASGFTFSSDAMNWVRQAPGKGLEWVAVIWNEGSNKYYADSVKGRFTISRDNSKNTLYLQMNSLRAEDTAVYYCARDRGPLWPLDYWGQGTLVTVSSASTKGPSVFPLAPSSKSTSGGTAALGCLVKDYFPEPVTVSWNSGALTSGVHTFPAVLQSSGLYSLSSVVTVPSSSLGTQTYICNVNHKPSNTKVDKKVEPKSCDKTHTCPPCPAPELLGGPSVFLFPPKPKDTLMISRTPEVTCVVVDVSHEDPEVKFNWYVDGVEVHNAKTKPREEQYNSTYRVVSVLTVLHQDWLNGKEYKCKVSNKALPAPIEKTISKAKGQPREPQVYTLPPSREEMTKNQVSLTCLVKGFYPSDIAVEWESNGQPENNYKTTPPVLDSDGSFFLYSKLTVDKSRWQQGNVFSCSVMHEALHNHYTQKSLSLSPGK

SEQ ID NO: 36 - protein, 449 aa, synthetic construct
  source 1..449: note = HC
QVQLVESGGGVVQPGRSLRLSCAASGFTFSSDAMNWVRQAPGKGLEWVAVIWNDASNKYYADSVKGRFTISRDNSKNTLYLQMNSLRAEDTAVYYCARDRGPLWPLDYWGQGTLVTVSSASTKGPSVFPLAPSSKSTSGGTAALGCLVKDYFPEPVTVSWNSGALTSGVHTFPAVLQSSGLYSLSSVVTVPSSSLGTQTYICNVNHKPSNTKVDKKVEPKSCDKTHTCPPCPAPELLGGPSVFLFPPKPKDTLMISRTPEVTCVVVDVSHEDPEVKFNWYVDGVEVHNAKTKPREEQYNSTYRVVSVLTVLHQDWLNGKEYKCKVSNKALPAPIEKTISKAKGQPREPQVYTLPPSREEMTKNQVSLTCLVKGFYPSDIAVEWESNGQPENNYKTTPPVLDSDGSFFLYSKLTVDKSRWQQGNVFSCSVMHEALHNHYTQKSLSLSPGK

SEQ ID NO: 37 - protein, 214 aa, synthetic construct
  source 1..214: note = LC
DIQMTQSPSTLSASVGDRVTITCRASQSISRWLAWYQQKPGKAPKLLIYKASSLESGVPSRFSGSGSGTEFTLTISNLQPDDFATFYCQQYNSYSRTFGQGTKVEIKRTVAAPSVFIFPPSDEQLKSGTASVVCLLNNFYPREAKVQWKVDNALQSGNSQESVTEQDSKDSTYSLSSTLTLSKADYEKHKVYACEVTHQGLSSPVTKSFNRGEC

SEQ ID NO: 38 - protein, 214 aa, synthetic construct
  source 1..214: note = LC
DIQMTQSPSTLSASVGDRVTITCRASQSISRWLAWYQQKPGKAPKLLIYKASSLESGVPSRFSGSGSGTEFTLTISNLQPDDFATFYCQQYSSYSRTFGQGTKVEIKRTVAAPSVFIFPPSDEQLKSGTASVVCLLNNFYPREAKVQWKVDNALQSGNSQESVTEQDSKDSTYSLSSTLTLSKADYEKHKVYACEVTHQGLSSPVTKSFNRGEC

SEQ ID NO: 39 - protein, 214 aa, synthetic construct
  source 1..214: note = LC
DIQMTQSPSTLSASVGDRVTITCRASQSISRWLAWYQQKPGKAPKLLIYKASSLESGVPSRFSGSGSGTEFTLTISNLQPDDFATFYCQQYNAYSRTFGQGTKVEIKRTVAAPSVFIFPPSDEQLKSGTASVVCLLNNFYPREAKVQWKVDNALQSGNSQESVTEQDSKDSTYSLSSTLTLSKADYEKHKVYACEVTHQGLSSPVTKSFNRGEC

SEQ ID NO: 40 - protein, 214 aa, synthetic construct
  source 1..214: note = LC
DIQMTQSPSTLSASVGDRVTITCRASQSISRWLAWYQQKPGKAPKLLIYKASSLESGVPSRFSGSGSGTEFTLTISNLQPDDFATFYCQQYQSYSRTFGQGTKVEIKRTVAAPSVFIFPPSDEQLKSGTASVVCLLNNFYPREAKVQWKVDNALQSGNSQESVTEQDSKDSTYSLSSTLTLSKADYEKHKVYACEVTHQGLSSPVTKSFNRGEC

SEQ ID NO: 41 - protein, 214 aa, synthetic construct
  source 1..214: note = LC
DIQMTQSPSTLSASVGDRVTITCRASQSISRWLAWYQQKPGKAPKLLIYKASSLESGVPSRFSGSGSGTEFTLTISNLQPDDFATFYCQQYNTYSRTFGQGTKVEIKRTVAAPSVFIFPPSDEQLKSGTASVVCLLNNFYPREAKVQWKVDNALQSGNSQESVTEQDSKDSTYSLSSTLTLSKADYEKHKVYACEVTHQGLSSPVTKSFNRGEC

SEQ ID NO: 42 - protein, 214 aa, synthetic construct
  source 1..214: note = LC
DIQMTQSPSTLSASVGDRVTITCRASQSISRWLAWYQQKPGKAPKLLIYKASSLESGVPSRFSGSGSGTEFTLTISNLQPDDFATFYCQQYTSYSRTFGQGTKVEIKRTVAAPSVFIFPPSDEQLKSGTASVVCLLNNFYPREAKVQWKVDNALQSGNSQESVTEQDSKDSTYSLSSTLTLSKADYEKHKVYACEVTHQGLSSPVTKSFNRGEC

SEQ ID NO: 43 - protein, 214 aa, synthetic construct
  source 1..214: note = LC
DIQMTQSPSTLSASVGDRVTITCRASQSISRWLAWYQQKPGKAPKLLIYKASSLESGVPSRFSGSGSGTEFTLTISNLQPDDFATFYCQQYASYSRTFGQGTKVEIKRTVAAPSVFIFPPSDEQLKSGTASVVCLLNNFYPREAKVQWKVDNALQSGNSQESVTEQDSKDSTYSLSSTLTLSKADYEKHKVYACEVTHQGLSSPVTKSFNRGEC

SEQ ID NO: 44 - protein, 25 aa, synthetic construct
  source 1..25: note = HFWR1
QVQLQESGPGLVKPSETLSLTCTVS

SEQ ID NO: 45 - protein, 10 aa, synthetic construct
  source 1..10: note = HCDR1
GGSINNYYWS

SEQ ID NO: 46 - protein, 14 aa, synthetic construct
  source 1..14: note = HFWR2
WVRQPPGKGLEWIG

SEQ ID NO: 47 - protein, 16 aa, synthetic construct
  source 1..16: note = HCDR2
YIFYSGSTNSNPSLKS

SEQ ID NO: 48 - protein, 32 aa, synthetic construct
  source 1..32: note = HFWR3
RVIISVDTSKNQFSLKLSSVTAADTAVYYCAR

SEQ ID NO: 49 - protein, 14 aa, synthetic construct
  source 1..14: note = HCDR3
EVGRIAVAGWFFDL

SEQ ID NO: 50 - protein, 11 aa, synthetic construct
  source 1..11: note = HFWR4
WGRGTLVTVSS

SEQ ID NO: 51 - protein, 23 aa, synthetic construct
  source 1..23: note = LFWR1
EIVMTQSPATLSVSPGERATLSC

SEQ ID NO: 52 - protein, 11 aa, synthetic construct
  source 1..11: note = LCDR1
RASQSVNSNLA

SEQ ID NO: 53 - protein, 15 aa, synthetic construct
  source 1..15: note = LFWR2
WYQQKPGQAPRLLIY

SEQ ID NO: 54 - protein, 7 aa, synthetic construct
  source 1..7: note = LCDR2
GASTRAT

SEQ ID NO: 55 - protein, 32 aa, synthetic construct
  source 1..32: note = LFWR3
GIPARFSGSGSGTEFTLTISSLQSEDFAVYYC

SEQ ID NO: 56 - protein, 9 aa, synthetic construct
  source 1..9: note = LCDR3
QQYNNWPLT

SEQ ID NO: 57 - protein, 10 aa, synthetic construct
  source 1..10: note = LFWR4
FGQGTRLEIK

SEQ ID NO: 58 - protein, 10 aa, synthetic construct
  source 1..10: note = HCDR1
GGSIQNYYWS

SEQ ID NO: 59 - protein, 16 aa, synthetic construct
  source 1..16: note = HCDR2
YIFYSGSTQSNPSLKS

SEQ ID NO: 60 - protein, 16 aa, synthetic construct
  source 1..16: note = HCDR2
YIFYSGSTNANPSLKS

SEQ ID NO: 61 - protein, 11 aa, synthetic construct
  source 1..11: note = LCDR1
RASQSVQSNLA

SEQ ID NO: 62 - protein, 11 aa, synthetic construct
  source 1..11: note = LCDR1
RASQSVNANLA

SEQ ID NO: 63 - protein, 122 aa, synthetic construct
  source 1..122: note = VH
QVQLQESGPGLVKPSETLSLTCTVSGGSINNYYWSWVRQPPGKGLEWIGYIFYSGSTNSNPSLKSRVIISVDTSKNQFSLKLSSVTAADTAVYYCAREVGRIAVAGWFFDLWGRGTLVTVSS

SEQ ID NO: 64 - protein, 122 aa, synthetic construct
  source 1..122: note = VH
QVQLQESGPGLVKPSETLSLTCTVSGGSIQNYYWSWVRQPPGKGLEWIGYIFYSGSTNSNPSLKSRVIISVDTSKNQFSLKLSSVTAADTAVYYCAREVGRIAVAGWFFDLWGRGTLVTVSS

SEQ ID NO: 65 - protein, 122 aa, synthetic construct
  source 1..122: note = VH
QVQLQESGPGLVKPSETLSLTCTVSGGSIQNYYWSWVRQPPGKGLEWIGYIFYSGSTQSNPSLKSRVIISVDTSKNQFSLKLSSVTAADTAVYYCAREVGRIAVAGWFFDLWGRGTLVTVSS

SEQ ID NO: 66 - protein, 122 aa, synthetic construct
  source 1..122: note = VH
QVQLQESGPGLVKPSETLSLTCTVSGGSIQNYYWSWVRQPPGKGLEWIGYIFYSGSTNANPSLKSRVIISVDTSKNQFSLKLSSVTAADTAVYYCAREVGRIAVAGWFFDLWGRGTLVTVSS

SEQ ID NO: 67 - protein, 107 aa, synthetic construct
  source 1..107: note = VL
EIVMTQSPATLSVSPGERATLSCRASQSVNSNLAWYQQKPGQAPRLLIYGASTRATGIPARFSGSGSGTEFTLTISSLQSEDFAVYYCQQYNNWPLTFGQGTRLEIK

SEQ ID NO: 68 - protein, 107 aa, synthetic construct
  source 1..107: note = VL
EIVMTQSPATLSVSPGERATLSCRASQSVQSNLAWYQQKPGQAPRLLIYGASTRATGIPARFSGSGSGTEFTLTISSLQSEDFAVYYCQQYNNWPLTFGQGTRLEIK

SEQ ID NO: 69 - protein, 107 aa, synthetic construct
  source 1..107: note = VL
EIVMTQSPATLSVSPGERATLSCRASQSVNANLAWYQQKPGQAPRLLIYGASTRATGIPARFSGSGSGTEFTLTISSLQSEDFAVYYCQQYNNWPLTFGQGTRLEIK

SEQ ID NO: 70 - protein, 452 aa, synthetic construct
  source 1..452: note = HC
QVQLQESGPGLVKPSETLSLTCTVSGGSINNYYWSWVRQPPGKGLEWIGYIFYSGSTNSNPSLKSRVIISVDTSKNQFSLKLSSVTAADTAVYYCAREVGRIAVAGWFFDLWGRGTLVTVSSASTKGPSVFPLAPSSKSTSGGTAALGCLVKDYFPEPVTVSWNSGALTSGVHTFPAVLQSSGLYSLSSVVTVPSSSLGTQTYICNVNHKPSNTKVDKKVEPKSCDKTHTCPPCPAPELLGGPSVFLFPPKPKDTLMISRTPEVTCVVVDVSHEDPEVKFNWYVDGVEVHNAKTKPREEQYNSTYRVVSVLTVLHQDWLNGKEYKCKVSNKALPAPIEKTISKAKGQPREPQVYTLPPSREEMTKNQVSLTCLVKGFYPSDIAVEWESNGQPENNYKTTPPVLDSDGSFFLYSKLTVDKSRWQQGNVFSCSVMHEALHNHYTQKSLSLSPGK

SEQ ID NO: 71 - protein, 452 aa, synthetic construct
  source 1..452: note = HC
QVQLQESGPGLVKPSETLSLTCTVSGGSIQNYYWSWVRQPPGKGLEWIGYIFYSGSTNSNPSLKSRVIISVDTSKNQFSLKLSSVTAADTAVYYCAREVGRIAVAGWFFDLWGRGTLVTVSSASTKGPSVFPLAPSSKSTSGGTAALGCLVKDYFPEPVTVSWNSGALTSGVHTFPAVLQSSGLYSLSSVVTVPSSSLGTQTYICNVNHKPSNTKVDKKVEPKSCDKTHTCPPCPAPELLGGPSVFLFPPKPKDTLMISRTPEVTCVVVDVSHEDPEVKFNWYVDGVEVHNAKTKPREEQYNSTYRVVSVLTVLHQDWLNGKEYKCKVSNKALPAPIEKTISKAKGQPREPQVYTLPPSREEMTKNQVSLTCLVKGFYPSDIAVEWESNGQPENNYKTTPPVLDSDGSFFLYSKLTVDKSRWQQGNVFSCSVMHEALHNHYTQKSLSLSPGK

SEQ ID NO: 72 - protein, 452 aa, synthetic construct
  source 1..452: note = HC
QVQLQESGPGLVKPSETLSLTCTVSGGSIQNYYWSWVRQPPGKGLEWIGYIFYSGSTQSNPSLKSRVIISVDTSKNQFSLKLSSVTAADTAVYYCAREVGRIAVAGWFFDLWGRGTLVTVSSASTKGPSVFPLAPSSKSTSGGTAALGCLVKDYFPEPVTVSWNSGALTSGVHTFPAVLQSSGLYSLSSVVTVPSSSLGTQTYICNVNHKPSNTKVDKKVEPKSCDKTHTCPPCPAPELLGGPSVFLFPPKPKDTLMISRTPEVTCVVVDVSHEDPEVKFNWYVDGVEVHNAKTKPREEQYNSTYRVVSVLTVLHQDWLNGKEYKCKVSNKALPAPIEKTISKAKGQPREPQVYTLPPSREEMTKNQVSLTCLVKGFYPSDIAVEWESNGQPENNYKTTPPVLDSDGSFFLYSKLTVDKSRWQQGNVFSCSVMHEALHNHYTQKSLSLSPGK

SEQ ID NO: 73 - protein, 452 aa, synthetic construct
  source 1..452: note = HC
QVQLQESGPGLVKPSETLSLTCTVSGGSIQNYYWSWVRQPPGKGLEWIGYIFYSGSTNANPSLKSRVIISVDTSKNQFSLKLSSVTAADTAVYYCAREVGRIAVAGWFFDLWGRGTLVTVSSASTKGPSVFPLAPSSKSTSGGTAALGCLVKDYFPEPVTVSWNSGALTSGVHTFPAVLQSSGLYSLSSVVTVPSSSLGTQTYICNVNHKPSNTKVDKKVEPKSCDKTHTCPPCPAPELLGGPSVFLFPPKPKDTLMISRTPEVTCVVVDVSHEDPEVKFNWYVDGVEVHNAKTKPREEQYNSTYRVVSVLTVLHQDWLNGKEYKCKVSNKALPAPIEKTISKAKGQPREPQVYTLPPSREEMTKNQVSLTCLVKGFYPSDIAVEWESNGQPENNYKTTPPVLDSDGSFFLYSKLTVDKSRWQQGNVFSCSVMHEALHNHYTQKSLSLSPGK

SEQ ID NO: 74 - protein, 214 aa, synthetic construct
  source 1..214: note = LC
EIVMTQSPATLSVSPGERATLSCRASQSVNSNLAWYQQKPGQAPRLLIYGASTRATGIPARFSGSGSGTEFTLTISSLQSEDFAVYYCQQYNNWPLTFGQGTRLEIKRTVAAPSVFIFPPSDEQLKSGTASVVCLLNNFYPREAKVQWKVDNALQSGNSQESVTEQDSKDSTYSLSSTLTLSKADYEKHKVYACEVTHQGLSSPVTKSFNRGEC

SEQ ID NO: 75 - protein, 214 aa, synthetic construct
  source 1..214: note = LC
EIVMTQSPATLSVSPGERATLSCRASQSVQSNLAWYQQKPGQAPRLLIYGASTRATGIPARFSGSGSGTEFTLTISSLQSEDFAVYYCQQYNNWPLTFGQGTRLEIKRTVAAPSVFIFPPSDEQLKSGTASVVCLLNNFYPREAKVQWKVDNALQSGNSQESVTEQDSKDSTYSLSSTLTLSKADYEKHKVYACEVTHQGLSSPVTKSFNRGEC

SEQ ID NO: 76 - protein, 214 aa, synthetic construct
  source 1..214: note = LC
EIVMTQSPATLSVSPGERATLSCRASQSVNANLAWYQQKPGQAPRLLIYGASTRATGIPARFSGSGSGTEFTLTISSLQSEDFAVYYCQQYNNWPLTFGQGTRLEIKRTVAAPSVFIFPPSDEQLKSGTASVVCLLNNFYPREAKVQWKVDNALQSGNSQESVTEQDSKDSTYSLSSTLTLSKADYEKHKVYACEVTHQGLSSPVTKSFNRGEC

SEQ ID NO: 77 - protein, 330 aa, synthetic construct
  source 1..330: note = recombinant cynomolgus MSLN ECD His-tag protein
DVERTTCPPEKEVHEIDESLIFYKKRELEACVDAALLAAQMDRVDAIPFTYEQLDVLKHKLDELYPQGYPESVIRHLGHLFLKMSPEDIRKWNVTSLETLKALLKVSKGHEMSAQVATLIDRVVVGRGQLDKDTVDTLTAFCPGCLCSLSPERLSSVPPSVIGAVRPQDLDTCGPRQLDVLYPKARLAFQNMSGSEYFVKIRPFLGGAPTEDVKALSQQNVSMDLATFMKLRREAVLPLTVAEVQKLLGPHVEGLKVEEQHSPVRDWILKQRQDDLDTLGLGLQGGIPNGYLILDLSVREALSGTPCLLGPGPVLTVLALLLASHHHHHH

SEQ ID NO: 78 - protein, 445 aa, synthetic construct
  source 1..445: note = HC
QVQLQESGPGLVKPSETLSLTCTVSGGSIFSHYWTWIRQFPGKGLEWIGYIYYSGSTNYNPSLKSRVTISVDTSKNQFSLKLSSVTAADTAVYYCARLGLGFDYWGQGSLVTVSSASTKGPSVFPLAPSSKSTSGGTAALGCLVKDYFPEPVTVSWNSGALTSGVHTFPAVLQSSGLYSLSSVVTVPSSSLGTQTYICNVNHKPSNTKVDKKVEPKSCDKTHTCPPCPAPELLGGPSVFLFPPKPKDTLMISRTPEVTCVVVDVSHEDPEVKFNWYVDGVEVHNAKTKPREEQYNSTYRVVSVLTVLHQDWLNGKEYKCKVSNKALPAPIEKTISKAKGQPREPQVYTLPPSREEMTKNQVSLTCLVKGFYPSDIAVEWESNGQPENNYKTTPPVLDSDGSFFLYSKLTVDKSRWQQGNVFSCSVMHEALHNHYTQKSLSLSPGK

SEQ ID NO: 79 - protein, 214 aa, synthetic construct
EIVMTQSPATLSVSPGERATLSCRASQSVNSNLAWYQQKPGQAPRLLIYGASTRATGIPARFSGSGSGTEFTLTISSLQSEDFAVYYCQQYFSWPYTFGQGTKLEIKRTVAAPSVFIFPPSDEQLKSGTASVVCLLNNFYPREAKVQWKVDNALQSGNSQESVTEQDSKDSTYSLSSTLTLSKADYEKHKVYACEVTHQGLSSPVTKSFNRGEC